European Patent Application EP 4 790 071 A2, published August 12, 2026. Title: Anti-CD73 antibody and use thereof. Applicant: Akeso Biopharma, Inc. Application EP, filed April 22, 2021. The sequence listing filed with the application follows.

SEQUENCE LISTING (22 sequences)

SEQ ID NO: 1 - DNA, 363 bp, synthetic construct
  misc_feature 1..363: note = Synthetic Artificial Sequence
  source 1..363: mol_type = other DNA
gaggtgcagctgcagcagtccggaccagagctggtgaagcctggcgcctccatgcggatgtcttgtaaggcctctggctacagcttcaccggctatacaatgaactgggtgaagcagtctcacggcaagaatctggagtggatcggcctgatcaacccttacaatgccggcaccagctataaccagaagtttaagggcaaggccaccctgacagtggacaagagctcctctaccgcctacatggagctgctgtccctgacatctgaggatagcgccgtgtactattgcgcccggtccgagtacagatatggcggcgactactttgattattggggccagggcaccacactgacagtgagctcc

SEQ ID NO: 2 - protein, 121 aa, synthetic construct
  REGION 1..121: note = Synthetic Artificial Sequence
EVQLQQSGPELVKPGASMRMSCKASGYSFTGYTMNWVKQSHGKNLEWIGLINPYNAGTSYNQKFKGKATLTVDKSSSTAYMELLSLTSEDSAVYYCARSEYRYGGDYFDYWGQGTTLTVSS

SEQ ID NO: 3 - DNA, 339 bp, synthetic construct
  misc_feature 1..339: note = Synthetic Artificial Sequence
  source 1..339: mol_type = other DNA
gacatcgtgatgacccagtctccaagctccctggcaatgagcgtgggacagaaggtgacaatgtcttgtaagtctagccagagcctgctgaactcctctaatcagaagaactacctggcctggtatcagcagaagccaggccagtctcccaagctgctggtgtactttgccagcaccagggagtccggagtgcctgacagattcatcggctccggctctggcacagacttcaccctgacaatcagctccgtgcaggcagaggacctggcagattatttctgccagcagcactacgacaccccttatacatttggcggcggcaccaagctggagatcaag

SEQ ID NO: 4 - protein, 113 aa, synthetic construct
  REGION 1..113: note = Synthetic Artificial Sequence
DIVMTQSPSSLAMSVGQKVTMSCKSSQSLLNSSNQKNYLAWYQQKPGQSPKLLVYFASTRESGVPDRFIGSGSGTDFTLTISSVQAEDLADYFCQQHYDTPYTFGGGTKLEIK

SEQ ID NO: 5 - DNA, 363 bp, synthetic construct
  misc_feature 1..363: note = Synthetic Artificial Sequence
  source 1..363: mol_type = other DNA
caggtgcagctgcagcagtctggagcagaggtggtgaagccaggagcctctatgaagatgagctgtaaggccagcggctactccttcaccggctatacaatgaactgggtgaagcaggcccacggccagaatctggagtggatcggcctgatcaacccttacaatgccggcacctcttataaccagaagtttcagggcaaggccaccctgacagtggacaagtccacctctacagcctacatggagctgagctccctgcggagcgaggatacagccgtgtactattgcgcccggtccgagtacagatatggcggcgactactttgattattggggccagggcaccacactgaccgtgtctagc

SEQ ID NO: 6 - protein, 121 aa, synthetic construct
  REGION 1..121: note = Synthetic Artificial Sequence
QVQLQQSGAEVVKPGASMKMSCKASGYSFTGYTMNWVKQAHGQNLEWIGLINPYNAGTSYNQKFQGKATLTVDKSTSTAYMELSSLRSEDTAVYYCARSEYRYGGDYFDYWGQGTTLTVSS

SEQ ID NO: 7 - DNA, 339 bp, synthetic construct
  misc_feature 1..339: note = Synthetic Artificial Sequence
  source 1..339: mol_type = other DNA
gacatcgtgatgacccagtccccaagctccctggcaatgtctgtgggagagagggtgacaatgtcctgtaagtctagccagtctctgctgaactcctctaatcagaagaactacctggcctggtatcagcagaagcccggccaggcccctaagctgctggtgtactttgcctctaccagggagagcggagtgccagacagattctctggcagcggctccggcacagacttcaccctgacaatcagctccgtgcaggcagaggacctggcagattatttctgccagcagcactacgataccccctatacatttggcggcggcaccaagctggagatcaag

SEQ ID NO: 8 - protein, 113 aa, synthetic construct
  REGION 1..113: note = Synthetic Artificial Sequence
DIVMTQSPSSLAMSVGERVTMSCKSSQSLLNSSNQKNYLAWYQQKPGQAPKLLVYFASTRESGVPDRFSGSGSGTDFTLTISSVQAEDLADYFCQQHYDTPYTFGGGTKLEIK

SEQ ID NO: 9 - DNA, 363 bp, synthetic construct
  misc_feature 1..363: note = Synthetic Artificial Sequence
  source 1..363: mol_type = other DNA
caggtgcagctggtgcagtctggagcagaggtggtgaagccaggagcctctgtgaaggtgagctgtaaggccagcggctactccttcaccggctatacaatgaactgggtgaggcaggcaccaggacagaatctggagtggatcggcctgatcaacccttacaatgccggcacctcttataaccagaagtttcagggcaaggtgaccctgacagtggacaagtccacctctacagcctacatggagctgagctccctgcggagcgaggatacagccgtgtactattgcgcccggtccgagtacagatatggcggcgactactttgattattggggccagggcaccacactgaccgtgtctagc

SEQ ID NO: 10 - protein, 121 aa, synthetic construct
  REGION 1..121: note = Synthetic Artificial Sequence
QVQLVQSGAEVVKPGASVKVSCKASGYSFTGYTMNWVRQAPGQNLEWIGLINPYNAGTSYNQKFQGKVTLTVDKSTSTAYMELSSLRSEDTAVYYCARSEYRYGGDYFDYWGQGTTLTVSS

SEQ ID NO: 11 - DNA, 339 bp, synthetic construct
  misc_feature 1..339: note = Synthetic Artificial Sequence
  source 1..339: mol_type = other DNA
gacatcgtgatgacccagtccccaagctccctggccgtgtctgtgggagagcgggtgacaatctcctgtaagtctagccagtctctgctgaactcctctaatcagaagaactacctggcctggtatcagcagaagcccggccaggcccctaagctgctgatctacttcgcctctaccagggagagcggagtgccagacagattctctggcagcggctccggcacagacttcaccctgacaatcagctccgtgcaggcagaggacgtggcagattactattgccagcagcactacgataccccctatacatttggcggcggcaccaagctggagatcaag

SEQ ID NO: 12 - protein, 113 aa, synthetic construct
  REGION 1..113: note = Synthetic Artificial Sequence
DIVMTQSPSSLAVSVGERVTISCKSSQSLLNSSNQKNYLAWYQQKPGQAPKLLIYFASTRESGVPDRFSGSGSGTDFTLTISSVQAEDVADYYCQQHYDTPYTFGGGTKLEIK

SEQ ID NO: 13 - DNA, 339 bp, synthetic construct
  misc_feature 1..339: note = Synthetic Artificial Sequence
  source 1..339: mol_type = other DNA
gacatcgtgatgacccagtccccaagctccctggccgtgtctgtgggagagcgggtgacaatctcctgtaagtctagccagtctctgctgaactcctctaatcagaagaactacctggcctggtatcagcagaagcccggccaggcccctaagctgctgatctacttcgcctctaccagggagagcggagtgccagacagattctctggcagcggctccggcacagacttcaccctgacaatcagctccctgcaggcagaggacgtggccgtgtactattgccagcagcactacgataccccctatacatttggcggcggcaccaagctggagatcaag

SEQ ID NO: 14 - protein, 113 aa, synthetic construct
  REGION 1..113: note = Synthetic Artificial Sequence
DIVMTQSPSSLAVSVGERVTISCKSSQSLLNSSNQKNYLAWYQQKPGQAPKLLIYFASTRESGVPDRFSGSGSGTDFTLTISSLQAEDVAVYYCQQHYDTPYTFGGGTKLEIK

SEQ ID NO: 15 - protein, 8 aa, synthetic construct
  REGION 1..8: note = Synthetic Artificial Sequence
GYSFTGYT

SEQ ID NO: 16 - protein, 8 aa, synthetic construct
  REGION 1..8: note = Synthetic Artificial Sequence
INPYNAGT

SEQ ID NO: 17 - protein, 14 aa, synthetic construct
  REGION 1..14: note = Synthetic Artificial Sequence
ARSEYRYGGDYFDY

SEQ ID NO: 18 - protein, 12 aa, synthetic construct
  REGION 1..12: note = Synthetic Artificial Sequence
QSLLNSSNQKNY

SEQ ID NO: 19 - skipped

SEQ ID NO: 20 - protein, 9 aa, synthetic construct
  REGION 1..9: note = Synthetic Artificial Sequence
QQHYDTPYT

SEQ ID NO: 21 - protein, 330 aa, synthetic construct
  REGION 1..330: note = Synthetic Artificial Sequence
ASTKGPSVFPLAPSSKSTSGGTAALGCLVKDYFPEPVTVSWNSGALTSGVHTFPAVLQSSGLYSLSSVVTVPSSSLGTQTYICNVNHKPSNTKVDKKVEPKSCDKTHTCPPCPAPEAAGGPSVFLFPPKPKDTLMISRTPEVTCVVVDVSHEDPEVKFNWYVDGVEVHNAKTKPREEQYNSTYRVVSVLTVLHQDWLNGKEYKCKVSNKALPAPIEKTISKAKGQPREPQVYTLPPSRDELTKNQVSLTCLVKGFYPSDIAVEWESNGQPENNYKTTPPVLDSDGSFFLYSKLTVDKSRWQQGNVFSCSVMHEALHNHYTQKSLSLSPGK

SEQ ID NO: 22 - protein, 107 aa, synthetic construct [sequence omitted]